European Patent Application EP 4 450 629 A1, published October 23, 2024. Title: Whooping Cough Antigen Recombinant Expression Vector, and Engineered Strain and Use thereof. Applicant: 远大赛威信生命科学（南京）有限公司. Application WO PCT/CN2022/131069, filed November 10, 2022. The sequence listing filed with the application follows.

SEQUENCE LISTING (26 sequences)

SEQ ID NO: 1 - DNA, 10773 bp, Bordetella pertussis
  source 1..10773: mol_type = genomic DNA
atgaacacgaacctgtacaggctggtcttcagccatgttcgcggcatgcttgttcccgtgagcgagcattgcaccgtcggaaacaccttctgtgggcgcacgcgtggtcaagcgcgaagtggggcccgcgccacgagcctgtccgtagcgcccaatgcgctggcctgggccctgatgttggcgtgtacgggtcttccgttagtaacgcacgcccagggcttggttcctcaggggcagacacaggtgctgcagggcgggaacaaggttcccgttgtcaatatcgccgacccaaattccggcggcgtctcgcacaacaagttccagcagttcaacgtcgccaaccctggcgtggtcttcaacaacggcctgaccgacggcgtgtccaggatcggcggggcgctgaccaagaaccccaacctgactcgccaggcctcggccattcttgccgaagtcacggacacttcgcccagtcgcctggccggtacgctcgaagtctatggcaagggcgccgacctcatcatcgccaaccccaacggcatcagcgtcaacggcctgagcacgctcaacgccagcaacctgacgctcacgacggggcgtcccagcgtcaacggcggccgcatcggccttgatgtccaacagggcaccgtcacgatcgaacgaggcggcgtcaatgccaccggcctgggctatttcgacgtggtggcgcgcctggtcaagctgcagggtgccgtgtcgagcaagcagggcaagcccctggccgacatcgcggtggtcgccggcgccaaccggtacgaccacgcaacccgccgcgccacgccgatcgccgcaggcgcgcgcggcgccgccgcgggcgcctacgcgattgacggcacggcggcgggcgccatgtacggcaagcacatcacgctggtgtccagcgattcaggcctgggcgtgcgccagctcggcagcctgtcctcgccatcggccatcaccgtgtcgtcgcagggcgaaatcgcgctgggcgacgccacggtccagcgcggcccgctcagcctcaagggcgcgggggtcgtgtcggccggcaaactggcctccggggggggggcggtgaacgtcgcgggcggcggggcggtgaagatcgcgtcggccagcagcgttggaaacctcgcggtgcaaggcggcggcaaggtacaggccacgctgttgaatgccggggggacgttgctggtgtcgggccgccaggccgtccagcttggcgcggcgagcagccgtcaggcgctgtccgtgaacgcgggcggcgccctcaaggcggacaagctgtcggcgacgcgacgggtcgacgtggatggcaagcaggccgtcgcgctggggtcggccagcagcaatgcgctgtcggtgcgtgccggcggcgccctcaaggcgggcaagctgtcggcgacggggcgactggacgtggacggcaagcaggccgtcacgctgggttcggttgcgagcgacggtgcgctgtcggtaagcgctggcggaaacctgcgggcgaagcaattggtctccagtgcccaacttgaggtgcgtgggcagcgggaggtcgcgctggatgacgcttcgagcgcacgcggcatgaccgtggttgccgcaggagcgctggcggcccgcaacctgcagtccaagggcgccatcggcgtacagggtggagaggcggtcagcgtggccaacgcgaacagcgacgcggaattgcgcgtgcgcgggcgcggccaggtggatctgcacgacctgagcgcagcgcgcggcgcggatatctccggcgaggggcgcgtcaatatcggccgtgcgcgcagcgatagcgatgtgaaggtctccgcgcacggcgccttgtcgatcgatagcatgacggccctcggtgcgatcggcgtccaggcaggcggcagcgtgtcggccaaggatatgcgcagccgtggcgccgtcaccgtcagcggcggcggcgccgtcaacctgggcgatgtccagtcggatgggcaggtccgcgccaccagcgcgggcgccatgacggtgcgagacgtcgcggctgccgccgaccttgcgctgcaggcgggcgacgcgttgcaggccgggttcctgaaatcggccggtgccatgaccgtgaacggccgcgatgccgtgcgactggatggcgcgcacgcgggcgggcaattgcgggtttccagcgacgggcaggctgcgttgggcagtctcgcggccaagggcgagctgacggtatcggccgcgcgcgcggcgaccgtggccgagttgaagtcgctggacaacatctccgtgacgggcggcgaacgcgtgtcggttcagagcgtcaacagcgcgtccagggtcgccatttcggcgcacggcgcgctggatgtaggcaaggtttccgccaagagcggtatcgggctcgaaggctggggcgcggtcggagcggactccctcggttccgacggcgcgatcagcgtgtccgggcgcgatgcggtcagggtcgatcaagcccgcagtcttgccgacatttcgctgggggcggaaggcggcgccacgctgggcgcggtggaggccgccggttcgatcgacgtgcgcggcggatccacggtggcggcgaactcgctgcacgccaatcgcgacgttcgggtcagcggcaaggatgcggtgcgcgtaacggccgccaccagcgggggcggtctgcatgtgtcgagcggccgccagctcgatctgggcgccgtgcaggcgcgcggcgcgctggccctggacggaggcgccggcgtggcgctgcaatcggccaaggctagcggcacgctgcatgtgcagggcggcgagcacctggacctgggcacgttggccgccgtaggggcggtggacgtcaatggcacgggagacgtgcgcgttgcgaagctggtgagcgatgcaggcgccgatctgcaagcggggcgctccatgacgctgggtatcgtcgacacgaccggcgatctgcaggcgcgcgcgcagcagaagctggagctcgggtcggttaagagcgatggcggccttcaggccgccgccggcggggccctcagcctggcggcggcggaagtcgcaggggcgctggagctctcgggccagggcgtcaccgtggacagagccagcgctagccgggcacgcatcgacagcaccggttcggtcggcatcggcgcgctgaaggcaggcgctgtcgaggccgcctcgccacggcgggcgcgccgcgcgctgcggcaggatttcttcacgcccggcagcgtggtggtccgcgcccagggcaatgtcacggtcgggcgcggcgatccgcatcagggcgtgctggcccagggcgacatcatcatggatgcgaagggcggcaccttgctgttgcgcaacgatgccttgaccgagaacgggacggtcaccatatcggccgattcggccgtgctcgagcattccaccatcgagagcaagatcagccagagcgtgctggctgccaaaggggacaagggcaagccggcggtgtcggtgaaggtcgcgaagaagctgtttctcaatggtacgttgcgggccgtcaacgacaacaacgaaaccatgtccgggcgccagatcgacgtcgtggacggacgtccgcagatcaccgacgcggtcacgggcgaagcgcgtaaggacgaatcggttgtgtccgacgccgcgctcgtggccgatggcggtccgatcgtggtcgaggccggcgagctggtcagccatgccggcggtatcggcaacggccgcaacaaggagaatggcgccagcgtcaccgtgcgcacgactggcaacctggtcaacaagggctacatctcggccggcaagcagggcgtgctcgaggtgggcggcgccttgacgaacgagttcctggtcggctcggacggcacccagcgcatcgaggcgcagcgcatcgagaacaggggcaccttccagagccaggctccggcgggcacggccggcgccctggtggtcaaggctgccgaggccatcgtgcacgacggcgtcatggccaccaaaggcgagatgcagatcgccggcaagggcggcgggtctccgaccgtcaccgccggcgcaaaggcgacgaccagcgcgaacaagctgagcgtcgacgtggcaagctgggacaacgcgggaagcctggatatcaagaagggcggcgcgcaggtcacggtggccgggcgctatgccgagcacggcgaggtttcgatacagggcgattacaccgtctcggccgacgccatcgcgctggcggcgcaggtcacccagcgcggaggcgccgcgaacctgacctcgcggcacgacacccgtttctccaacaagattcgcctgatggggccgttgcaggtcaacgccggcggcgcggtgtccaataccggcaatctgaaagtgcgcgagggcgtgaccgtaacggcggcgtcgttcgacaacgagaccggggccgaggtcatggccaagagcgccacgctgacgacttccggggccgcgcgcaacgcgggcaagatgcaggtcaaggaggccgccacgatcgttgccgccagcgtttccaatcccggcacgttcacggccggcaaggatatcactgttacctcgcgcggaggattcgataacgaaggcaagatggagtccaacaaggacatcgtcatcaagacggaacagttcagcaatggcagggttctcgacgccaagcatgatctgacggtcacggcgagcgggcaggcggacaaccggggcagcctgaaggcaggccacgatttcacggtgcaggcccagcgtatcgacaatagcggaaccatggccgccggccacgacgccacgctgaaggcgccgcacctgcgcaatacgggccaggtcgtagccgggcacgacatccatatcatcaacagcgccaagctggagaacaccgggcgcgtggatgcgcgcaacgacatcgctctggatgtggcggatttcaccaacacgggatccctctacgccgagcatgacgcgacgctgacgcttgcgcaaggcacgcagcgcgatctggtggtggaccaggatcatatcctgccggtggcggaggggacgttacgcgtcaaggccaagtcgctgaccaccgaaatcgagaccggcaatcccggcagcctgatcgccgaggtgcaggaaaatatcgacaacaagcaggccatcgtcgtcggcaaggacctgacgctgagttcggcgcacggcaacgtggccaacgaagcgaacgcgctgctgtgggccgccggggagctgaccgtcaaggcgcagaacatcaccaataaacgggccgcgctgatcgaggcgggcggcaacgcccggctgacggcggccgttgccttgctcaacaagctgggccgcattcgcgcgggcgaggacatgcacctggatgcgccgcgcatcgagaacaccgcgaaactgagcggcgaggtgcaacgcaaaggcgtgcaggacgtcgggggaggcgagcacggccgctggagcggtatcggctatgtcaactactggttgcgcgccggcaatgggaagaaggcgggaaccatcgccgcgccgtggtatggcggtgatctgacggcggagcagtcgctcatcgaggtcggcaaggatctctatctgaatgccggagcgcgcaaggacgaacatcgccatctgctcaatgaaggcgtgatccaggcgggcggccatggccacatcggcggcgacgtggacaaccggtcggtggtgcgcaccgtgtccgccatggagtatttcaagacgcctcttccggtgagcctgactgccctggacaatcgtgccggcttgtctccggcgacctggaacttccagtccacgtatgaactcctggattatctgctggaccagaatcgctacgagtacatttgggggctgtatccgacctacaccgaatggtcggtgaatacgctgaagaacctcgacctgggctaccaggccaagccggctcccactgcgccgccgatgcccaaggctcccgaactcgacctgcgtggccatacgctggagtcggccgaaggccggaagatctttggcgagtacaagaagctgcaaggcgagtacgagaaggcgaagatggccgtccaggccgtggaggcttacggcgaggctactcggcgcgtccatgatcagctgggccaacgttatggtaaggccctgggcggcatggatgccgagaccaaggaggtcgacggcatcatccaggagttcgccgcggatctgcgaacggtctatgcgaagcaggccgaccaggcgaccatcgacgcagagacggacaaggtcgcccagcgctacaagtcgcagatcgacgcggtgcggctgcaggcgatccagcctggccgggtcacgctggccaaggcgctgtcggcggcgctgggcgccgactggcgcgcgctgggtcactcccaattgatgcagcgctggaaggatttcaaggcgggcaagcgcggcgcggaaatcgcgttctatcccaaggaacaaaccgtgctggccgccggcgccggtttgaccctgtccaacggggcgatccacaacggcgagaacgccgcgcagaatcgcggccggccggaaggcctgaaaatcggcgcacattcggcgacttcggtgagcggctcgttcgacgccttgcgcgacgtggggctggaaaagcggctggatatcgacgatgcgctggctgccgtgctcgtgaatccgcatattttcacgcggatcggggcggctcagacatcccttgccgacggcgccgccgggccggcgctggcgcgccaggccaggcaagcgccggagaccgacggcatggtggatgcgcgagggctgggcagcgccgatgcgctcgcttccctggccagcttggacgcggcgcaagggctggaggtatccggcaggcgcaatgcgcaggtggccgacgccgggctcgccgggccgagcgccgtcgcggcgccggccgtcggggcggccgatgtcggcgtggagcctgtcacgggggaccaggtcgaccagcctgtcgtggcggtcgggctcgagcagcctgtcgcgacggtccgggtcgcgccgccagccgtcgcgttgccgcggccgctgttcgaaacccgcatcaagtttatcgaccagagcaaattctacggctcgcgttatttcttcgagcagatcggctacaagcccgatcgcgccgcgcgggtggcgggcgacaactatttcgataccacgctggtgcgcgagcaggtgcggcgcgccctgggcggctatgaaagccgcctgcccgtgcgcggtgtcgcgttggtggccaagctgatggattcggccgggacggtcggcaaggcgctgggcctgaaggtgggtgtcgcgccgaccgcgcagcagctcaagcaggccgaccgcgatttcgtctggtacgtggataccgtgatcgacggccagaaggttctcgctccccggctgtacctgaccgaggcgacgcgccagggcatcacggatcagtacgccggcggcggggcgctgattgcctccggcggcgacgtaactgtcaatacggacggccatgacgtcagttcggtcaacgggctgatccagggcaggagcgtcaaggtggacgcgggcaagggcaaggtcgtggtggccgacagcaagggggcgggcggcggcatcgaggccgatgacgaggtcgacgtctcaggccgggatatcggcatcgagggcggcaagctgcgcggcaaggatgtcaggctcaaggccgacacggtcaaggtcgcgacctcgatgcgttacgacgacaagggcaggctggcggcgcgcggcgacggcgccctggatgcgcaaggcggccagctgcatatcgaggccaagcgcctggagacggccggcgcgacgctcaagggcggcaaggtgaagctggatgtcgatgacgtcaagttgggcggcgtgtacgaggcggggtccagctacgagaacaagagctcgacgccgctgggcagcctgttcgccatcctgtcgtcgacgacggaaaccaaccagtcggcacacgcgaaccattacggtacgcgcatcgaagccggtacgctggaaggaaagatgcagaacctggagatcgaaggcggttcggtcgatgccgcgcatacggacctgtccgtggcccgcgacgcgaggttcaaggccgccgcggatttcgcgcacgccgagcatgagaaggatgtgcgccaactgtccctgggtgccaaggtgggggcgggcggctacgaggcgggcttcagcctgggcagcgaaagcggtctggaagcgcacgccggccgcggtatgaccgcgggcgctgaagtcaaggtaggttatcgggcatcgcacgaacagtcctcggaaaccgaaaagtcctatcgcaacgcgaacctcaatttcggtggaggctccgtcgaggctggcaatgtcctggatatcggcggcgccgacatcaaccggaaccggtacggcggcgccgcgaaggggaacgccgggaccgaggaggccttgcgcatgcgcgccaagaaggtcgagtccaccaagtacgtcagcgagcagacgagccagagctccggctggagcgtggaggtggcatcgacggccagtgcccgttccagcctgctgacggccgccacgcgcctgggcgacagcgtggcgcagaatgtcgaggacggccgcgagatccgcggcgagctgatggctgcgcaagtcgccgcggaggccacgcaactggtaaccgccgacacggcggcggtggcactgagtgccggaatcagcgccgacttcgacagcagccacagccgctccacctcgcagaatacccaatatctgggcggaaacttgtccatcgaggccaccgagggcgatgcgacgctggtgggcgcgaagttcggcggtggcgaccaggtcagcttgaaggcagcgaagagcgtgaacctcatggcggccgaatcgaccttcgaatcgtactcggagagccacaacttccacgcctccgccgacgcgaaccttggcgccaacgccgtgcagggcgccgttggcctggggttgactgcgggtatggggacgtcgcatcagattaccaacgaaaccggcaagacctatgccggaacctcggtggatgcggcgaacgtgtcgatcgatgcaggcaaggatctgaacctttccgggtcccgcgtgcggggtaagcatgttgtcctggatgtcgagggcgatatcaatgcgaccagcaagcaggatgaacgcaactacaactccagcggtggcggttgggacgcctcggcaggggtggcgattcagaaccgcacgttggttgcgcccgtggggtctgccggcttcaatttcaatacggaacacgacaattcgcgcctgaccaatgacggggcggcgggtgtcgttgccagcgacgggttgacgggccatgtgaaaggcgacgccaacctgaccggcgcgaccattgccgatttgtcgggcaagggcaatctcaaggtcgacggcgcggtcaacgcgcagaacctgaaagactaccgcgacaaggacggcggcagcggcggcctgaacgtgggcatctcgtcgaccacgctggcgcccaccgtgggcgtggcgttcggcagggtggccggagaggattatcaggccgagcagcgcgccacgattgacgtcggtcaaaccaaggatcccgcgcgcctgcaggtcggcggcggcgtcaagggtaccctcaatcaggacgccgcgcaggccacggtcgttcagcgcaacaagcactgggccggaggcgggtcggaattctcggtggctggcaagtcactgaagaagaagaaccaggtccgcccggtggagacgccgacgccggatgtcgtggatggaccgcctagccgtcccaccacgccgcccgcgtcgccgcagccgatccgcgcgacggtcgaggtcagttcgccgccgccggtgtccgtggccacggtcgaagtcgtgccgcggccgaaggtcgaaacggctcagccgcttccgcctcggccggtggcggcccaggtcgtgccggtgacgcctcccaaggtggaggtcgccaaggtggaagtcgtgccgcggccgaaggttgaaacggctcagccgcttccgccccggccggtggtggccgagaaggtgacgacgccggcggtccagccccagcttgccaaggtggagacggtgcagccggtgaagcccgaaaccaccaagccgttgcccaagccgctgccggtggcgaaggtgacgaaagcgccgccgccggttgtggagaccgcccagccgctgccgccggtcaagccacagaaggcgacccccggccccgtggctgaggtgggcaaggctacggtcacgacggtgcaggtgcagagtgcgccgcccaagccggccccggtggccaagcagcccgcgcctgcaccgaagcccaagcccaagcccaagcccaaggccgagcgtccgaagccgggcaaaacgacgcccttgagcgggcgccacgtggtgcaacagcaggtgcaggtcttgcagcggcaagcgagtgacatcaacaacaccaagagcctgcctggcgggaagctgcccaagccggtcaccgtgaagctgaccgacgagaacggcaagccgcagacgtatacgatcaaccggcgcgaggatctgatgaagctcaacggcaaggtgctgtccaccaagacgacactgggcctggagcagaccttccgcctgcgggtcgaggatatcggcggcaagaactaccgggtcttctatgaaaccaacaaatag

SEQ ID NO: 2 - DNA, 1000 bp, synthetic construct
  source 1..1000: mol_type = other DNA
tcagcttctgcagcaggcgcgtcttgtaggtgctgacggtcttgttgctgaggaacatgctgtcagcgatgtccttgttggacatgccttgcgccagcagttgcaggacggtcagttcgcggttggacaacacgctgatgagcgtactgtcgctcttggcgttgtcgcccatgcgcatctcgctgagcgtggtgctggggaagtaggtgtagccggccatcaccgccttggcggcattgatgacctcgtgcaggttctcgtgtttgcacacgaagcctgcggcgccggagttcaggcagcggcgggcgaacagcgaaggcggctggccggtcagcaccagcacgcgtagcggcaaccccagcgattgcagccgggcgatgacttccagcccgtccagcttgggaatgccgatgtcgagtacgacgaggttgggaattttctcgcgggcgatcttgagcccgtcaatgccgttatcggtttcgccgatgacttcgaatccttccttttccatcaggacccggacggcgaatctcagtacagggtgatcgtcaatgatgaggactttgttgtacatgataagaagaatatgctttgagtttcgtggcgagaaaaaaatcctgcaacgcgtaatgtcattgatgcgtcaaaggaatggctgcgaaatttcacattctcctatacgtcagcaagcaacgatacgggcatgagtgctgctaaacagtatcctataccaaaataggaaaagtctgaattcctgcgctggcacccgcggcgggccggggagcgggttgtcggcgcacgcctatacgtgccggacagggtttgatggtttgactaagaaatttcctacaagtcttgtataaatatccattgatggacgggatcattactgactgacgaagtgctgaggtttatccagactatggcactggatttcaaaacctaaaacgagcaggccgataacggattctgccgattacttcacttcgctggtcggaat

SEQ ID NO: 3 - DNA, 2733 bp, Bordetella pertussis
  source 1..2733: mol_type = genomic DNA
atgaacatgtctctgtcacgcattgtcaaggcggcgcccctgcgccgcaccacgctggccatggcgctgggcgcgctgggcgccgccccggcggcgcatgccgactggaacaaccagtccatcgtcaagaccggtgagcgccagcatggcatccatatccagggctccgacccgggcggcgtacggaccgccagcggaaccaccatcaaggtaagcggccgtcaggcccagggcatcctgctagaaaatcccgcggccgagctgcagttccggaacggcagtgtcacgtcgtcgggacagttgtccgacgatggcatccggcgctttctgggcaccgtcaccgtcaaggccggcaagctggtcgccgatcacgccacgctggccaacgttggcgacacctgggacgacgacggcatcgcgctctatgtggccggcgaacaggcccaggccagcatcgccgacagcaccctgcagggcgctggcggcgtgcagatcgagcgcggcgccaatgtcacggtccaacgcagcgccatcgtcgacgggggcttgcatatcggcgccctgcagtcattgcagccggaagaccttccgcccagccgggtggtgctgcgcgacaccaacgtgaccgccgtgcccgccagcggcgcgcccgcggcggtgtctgtgttgggggccagtgagcttacgctcgacggcgggcacatcaccggcgggcgggcagcgggggtggcggccatgcaaggggcggtcgtgcatctgcagcgcgcgacgatacggcgcggggacgcgcctgccggcggtgcggttcccggcggtgcggttcccggtggtgcggttcccggcggcttcggtcccggcggcttcggtcccgtcctcgacggctggtatggcgtggacgtatcgggctccagcgtggagctcgcccagtcgatcgtcgaggcgccggagctgggcgccgcaatccgggtgggccgcggcgccagggtgacggtgtcgggcggcagcttgtccgcaccgcacggcaatgtcatcgagaccggcggcgcgcgtcgctttgcgcctcaagccgcgcccctgtcgatcaccttgcaggccggcgcgcatgcccaggggaaagcgctgctgtaccgggtcctgccggagcccgtgaagctgacgctgaccgggggcgccgatgcgcagggcgacatcgtcgcgacggagctgccctccattcccggcacgtcgatcgggccgctcgacgtggcgctggccagccaggcccgatggacgggcgctacccgcgcggtcgactcgctgtccatcgacaacgccacctgggtcatgacggacaactcgaacgtcggtgcgctacggctggccagcgacggcagcgtcgatttccagcagccggccgaagctgggcggttcaaggtcctgacggtcaatacgctggcgggttcggggctgttccgcatgaatgtcttcgcggacctggggctgagcgacaagctggtcgtcatgcaggacgccagcggccagcacaggctgtgggtccgcaacagcggcagcgagccggccagcgccaacaccctgctgctggtgcagacgccactaggcagcgcggcgacctttacccttgccaacaaggacggcaaggtcgatatcggtacctatcgctatcgattggccgccaacggcaatgggcagtggagcctggtgggcgcgaaggcgccgccggcgcccaagcccgcgccgcagccgggtccccagccgccgcagccgccgcagccgcagccggaagcgccggcgccgcaaccgccggcgggcagggagttgtccgccgccgccaacgcggcggtcaacacgggtggggtgggcctggccagcacgctctggtacgccgaaagcaatgcgttgtccaagcgcctgggcgagttgcgcctgaatccggacgccggcggcgcctggggccgcggcttcgcgcaacgccagcagctggacaaccgcgccgggcggcgcttcgaccagaaggtggccggcttcgagctgggcgccgaccacgcggtggcggtggccggcggacgctggcacctgggcgggctggccggctatacgcgcggcgaccgcggcttcaccggcgacggcggcggccacaccgacagcgtgcatgtcgggggctatgccacatatatcgccgacagcggtttctacctggacgcgacgctgcgcgccagccgcctggagaatgacttcaaggtggcgggcagcgacgggtacgcggtcaagggcaagtaccgcacccatggggtgggcgcctcgctcgaggcgggccggcgctttacccatgccgacggctggttcctcgagccgcaggccgagctggcggtattccgggccggcggcggtgcgtaccgcgcggccaacggcctgcgggtgcgcgacgaaggcggcagctcggtgctgggtcgcctgggcctggaggtcggcaagcgcatcgaactggcaggcggcaggcaggtgcagccatacatcaaggccagcgtgctgcaggagttcgacggcgcgggtacggtacacaccaacggcatcgcgcaccgcaccgaactgcgcggcacgcgcgccgaactgggcctgggcatggccgccgcgctgggccgcggccacagcctgtatgcctcgtacgagtactccaagggcccgaagctggccatgccgtggaccttccacgcgggctaccggtacagctggtaa

SEQ ID NO: 4 - DNA, 1000 bp, synthetic construct
  source 1..1000: mol_type = other DNA
cattccaccatcgagagcaagatcagccagagcgtgctggctgccaaaggggacaagggcaagccggcggtgtcggtgaaggtcgcgaagaagctgtttctcaatggtacgttgcgggccgtcaacgacaacaacgaaaccatgtccgggcgccagatcgacgtcgtggacggacgtccgcagatcaccgacgcggtcacgggcgaagcgcgtaaggacgaatcggttgtgtccgacgccgcgctcgtggccgatggcggtccgatcgtggtcgaggccggcgagctggtcagccatgccggcggtatcggcaacggccgcaacaaggagaatggcgccagcgtcaccgtgcgcacgactggcaacctggtcaacaagggctacatctcggccggcaagcagggcgtgctcgaggtgggcggcgccttgacgaacgagttcctggtcggctcggacggcacccagcgcatcgaggcgcagcgcatcgagaacaggggcaccttccagagccaggctccggcgggcacggccggcgccctggtggtcaaggctgccgaggccatcgtgcacgacggcgtcatggccaccaaaggcgagatgcagatcgccggcaagggcggcgggtctccgaccgtcaccgccggcgcaaaggcgacgaccagcgcgaacaagctgagcgtcgacgtggcaagctgggacaacgcgggaagcctggatatcaagaagggcggcgcgcaggtcacggtggccgggcgctatgccgagcacggcgaggtttcgatacagggcgattacaccgtctcggccgacgccatcgcgctggcggcgcaggtcacccagcgcggaggcgccgcgaacctgacctcgcggcacgacacccgtttctccaacaagattcgcctgatggggccgttgcaggtcaacgccggcggcgcggtgtccaataccggcaatctgaaagtgcgcgagggcgtgaccgtaacggcggcgtcgttcgaca

SEQ ID NO: 5 - DNA, 933 bp, synthetic construct
  source 1..933: mol_type = other DNA
ccggaattgccagctggggcgccctctggtaaggttgggaagccctgcaaagtaaactggatggctttctcgccgccaaggatctgatggcgcaggggatcaagctctgatcaagagacaggatgaggatcgtttcgcatgattgaacaagatggattgcacgcaggttctccggccgcttgggtggagaggctattcggctatgactgggcacaacagacaatcggctgctctgatgccgccgtgttccggctgtcagcgcaggggcgcccggttctttttgtcaagaccgacctgtccggtgccctgaatgaactgcaagacgaggcagcgcggctatcgtggctggccacgacgggcgttccatgcgcagctgtgctcgacgttgtcactgaagcgggaagagactggctgctattgggcgaagtgccggggcaggatctcctgtcatctcaccttgctcctgccgagaaagtatccatcatggctgatgcaatgcggcggctgcatacgcttgatccggctacctgcccattcgaccaccaagcgaaacatcgcatcgagcgagcacgtactcggatggaagccggtcttgtcgatcaggatgatctggacgaagagcatcaggggctcgcgccagccgaactgttcgccaggctcaaggcgagcatgcccgacggcgaggatctcgtcgtgacccatggcgatgcctgcttgccgaatatcatggtggaaaatggccgcttttctggattcatcgactgtggccggctgggtgtggcggaccgctatcaggacatagcgttggctacccgtgatattgctgaagagcttggcggcgaatgggctgaccgcttcctcgtgctttacggtatcgccgctcccgattcgcagcgcatcgccttctatcgccttcttgacgagttcttctga

SEQ ID NO: 6 - DNA, 1275 bp, synthetic construct
  source 1..1275: mol_type = other DNA
atgtccaccaacttatcagtgataaagaatccgcgcgttcaatcggaccagcggaggctggtccggaggccagacatgaaacccaacatacccctgatcgtaattctgagcactgtcgcgctcgacgctgtcggcatcggcctgattatgccggtgctgccgggcctcctgcgcgatctggttcactcgaacgacgtcaccgcccactatggcattctgctggcgctgtatgcgttggtgcaatttgcctgcgcacctgtgctgggcgcgctgtcggatcgtttcgggcggcggccaatcttgctcgtctcgctggccggcgccactgtcgactacgccatcatggcgacagcgcctttcctttgggttctctatatcgggcggatcgtggccggcatcaccggggcgactggggcggtagccggcgcttatattgccgatatcactgatggcgatgagcgcgcgcggcacttcggcttcatgagcgcctgtttcgggttcgggatggtcgcgggacctgtgctcggtgggctgatgggcggtttctccccccacgctccgttcttcgccgcggcagccttgaacggcctcaatttcctgacgggctgtttccttttgccggagtcgcacaaaggcgaacgccggccgttacgccgggaggctctcaacccgctcgcttcgttccggtgggcccggggcatgaccgtcgtcgccgccctgatggcggtcttcttcatcatgcaacttgtcggacaggtgccggccgcgctttgggtcattttcggcgaggatcgctttcactgggacgcgaccacgatcggcatttcgcttgccgcatttggcattctgcattcactcgcccaggcaatgatcaccggccctgtagccgcccggctcggcgaaaggcgggcactcatgctcggaatgattgccgacggcacaggctacatcctgcttgccttcgcgacacggggatggatggcgttcccgatcatggtcctgcttgcttcgggtggcatcggaatgccggcgctgcaagcaatgttgtccaggcaggtggatgaggaacgtcaggggcagctgcaaggctcactggcggcgctcaccagcctgacctcgatcgtcggacccctcctcttcacggcgatctatgcggcttctataacaacgtggaacgggtgggcatggattgcaggcgctgccctctacttgctctgcctgccggcgctgcgtcgcgggctttggagcggcgcagggcaacgagccgatcgctga

SEQ ID NO: 7 - DNA, 966 bp, synthetic construct
  source 1..966: mol_type = other DNA
cgcggaacccctatttgtttatttttctaaatacattcaaatatgtatccgctcatgagacaataaccctgataaatgcttcaataatattgaaaaaggaagagtatgagtattcaacatttccgtgtcgcccttattcccttttttgcggcattttgccttcctgtttttgctcacccagaaacgctggtgaaagtaaaagatgctgaagatcagttgggtgcacgagtgggttacatcgaactggatctcaacagcggtaagatccttgagagttttcgccccgaagaacgttttccaatgatgagcacttttaaagttctgctatgtggcgcggtattatcccgtattgacgccgggcaagagcaactcggtcgccgcatacactattctcagaatgacttggttgagtactcaccagtcacagaaaagcatcttacggatggcatgacagtaagagaattatgcagtgctgccataaccatgagtgataacactgcggccaacttacttctgacaacgatcggaggaccgaaggagctaaccgcttttttgcacaacatgggggatcatgtaactcgccttgatcgttgggaaccggagctgaatgaagccataccaaacgacgagcgtgacaccacgatgcctgtagcaatggcaacaacgttgcgcaaactattaactggcgaactacttactctagcttcccggcaacaattaatagactggatggaggcggataaagttgcaggaccacttctgcgctcggcccttccggctggctggtttattgctgataaatctggagccggtgagcgtgggtctcgcggtatcattgcagcactggggccagatggtaagccctcccgtatcgtagttatctacacgacggggagtcaggcaactatggatgaacgaaatagacagatcgctgagataggtgcctcactgattaagcattggtaa

SEQ ID NO: 8 - DNA, 763 bp, synthetic construct
  source 1..763: mol_type = other DNA
tgatcggcacgtaagaggttccaactttcaccataatgaaataagatcactaccgggcgtattttttgagttatcgagattttcaggagctaaggaagctaaaatggagaaaaaaatcactggatataccaccgttgatatatcccaatggcatcgtaaagaacattttgaggcatttcagtcagttgctcaatgtacctataaccagaccgttcagctggatattacggcctttttaaagaccgtaaagaaaaataagcacaagttttatccggcctttattcacattcttgcccgcctgatgaatgctcatccggaattccgtatggcaatgaaagacggtgagctggtgatatgggatagtgttcacccttgttacaccgttttccatgagcaaactgaaacgttttcatcgctctggagtgaataccacgacgatttccggcagtttctacacatatattcgcaagatgtggcgtgttacggtgaaaacctggcctatttccctaaagggtttattgagaatatgtttttcgtctcagccaatccctgggtgagtttcaccagttttgatttaaacgtggccaatatggacaacttcttcgcccccgttttcaccatgggcaaatattatacgcaaggcgacaaggtgctgatgccgctggcgattcaggttcatcatgccgtctgtgatggcttccatgtcggcagaatgcttaatgaattacaacagtactgcgatgagtggcagggcggggcgtaa

SEQ ID NO: 9 - protein, 910 aa, Bordetella pertussis
MNMSLSRIVKAAPLRRTTLAMALGALGAAPAAHADWNNQSIVKTGERQHGIHIQGSDPGGVRTASGTTIKVSGRQAQGILLENPAAELQFRNGSVTSSGQLSDDGIRRFLGTVTVKAGKLVADHATLANVGDTWDDDGIALYVAGEQAQASIADSTLQGAGGVQIERGANVTVQRSAIVDGGLHIGALQSLQPEDLPPSRVVLRDTNVTAVPASGAPAAVSVLGASELTLDGGHITGGRAAGVAAMQGAVVHLQRATIRRGDAPAGGAVPGGAVPGGAVPGGFGPGGFGPVLDGWYGVDVSGSSVELAQSIVEAPELGAAIRVGRGARVTVSGGSLSAPHGNVIETGGARRFAPQAAPLSITLQAGAHAQGKALLYRVLPEPVKLTLTGGADAQGDIVATELPSIPGTSIGPLDVALASQARWTGATRAVDSLSIDNATWVMTDNSNVGALRLASDGSVDFQQPAEAGRFKVLTVNTLAGSGLFRMNVFADLGLSDKLVVMQDASGQHRLWVRNSGSEPASANTLLLVQTPLGSAATFTLANKDGKVDIGTYRYRLAANGNGQWSLVGAKAPPAPKPAPQPGPQPPQPPQPQPEAPAPQPPAGRELSAAANAAVNTGGVGLASTLWYAESNALSKRLGELRLNPDAGGAWGRGFAQRQQLDNRAGRRFDQKVAGFELGADHAVAVAGGRWHLGGLAGYTRGDRGFTGDGGGHTDSVHVGGYATYIADSGFYLDATLRASRLENDFKVAGSDGYAVKGKYRTHGVGASLEAGRRFTHADGWFLEPQAELAVFRAGGGAYRAANGLRVRDEGGSSVLGRLGLEVGKRIELAGGRQVQPYIKASVLQEFDGAGTVHTNGIAHRTELRGTRAELGLGMAAALGRGHSLYASYEYSKGPKLAMPWTFHAGYRYSW

SEQ ID NO: 10 - protein, 1083 aa, Bordetella pertussis
MRCTRAIRQTARTGWLTWLAILAVTAPVTSPAWADDPPATVYRYDSRPPEDVFQNGFTAWGNNDNVLDHLTGRSCQVGSSNSAFVSTSSSRRYTEVYLEHRMQEAVEAERAGRGTGHFIGYIYEVRADNNFYGAASSYFEYVDTYGDNAGRILAGALATYQSEYLAHRRIPPENIRRVTRVYHNGITGETTTTEYSNARYVSQQTRANPNPYTSRRSVASIVGTLVRMAPVIGACMARQAESSEAMAAWSERAGEAMVLVYYESIAYSFMPIDRKTLCHLLSVLPLALLGSHVARASTPGIVIPPQEQITQHGGPYGRCANKTRALTVAELRGSGDLQEYLRHVTRGWSIFALYDGTYLGGEYGGVIKDGTPGGAFDLKTTFCIMTTRNTGQPATDHYYSNVTATRLLSSTNSRLCAVFVRSGQPVIGACTSPYDGKYWSMYSRLRKMLYLIYVAGISVRVHVSKEEQYYDYEDATFETYALTGISICNPGSSLCMLRRFPTRTTAPGQGGARRSRVRALAWLLASGAMTHLSPALADVPYVLVKTNMVVTSVAMKPYEVTPTRMLVCGIAAKLGAAASSPDAHVPFCFGKDLKRPGSSPMEVMLRAVFMQQRPLRMFLGPKQLTFEGKPALELIRMVECSGKQDCPMKSPRRACWSAASPPNWAPRPAARTRTCRSASARISSVPAAVPWKSCCAPSSCNNGRCACFWVPSNSLSKASPRSNMQRQAGLPLKANPMHTIASILLSVLGIYSPADVAGLPTHLYKNFTVQELALKLKGKNQEFCLTAFMSGRSLVRACLSDAGHEHDTWFDTMLGFAISAYALKSRIALTVEDSPYPGTPGDLLELQICPLNGYCEMLINNKKLLHHILPILVLALLGMRTAQAVAPGIVIPPKALFTQQGGAYGRCPNGTRALTVAELRGNAELQTYLRQITPGWSIYGLYDGTYLGQAYGGIIKDAPPGAGFIYRETFCITTIYKTGQPAADHYYSKVTATRLLASTNSRLCAVFVRDGQSVIGACASPYEGRYRDMYDALRRLLYMIYMSGLAVRVHVSKEEQYYDYEDATFQTYALTGISLCNPAASIC

SEQ ID NO: 11 - DNA, 39 bp, synthetic construct
  source 1..39: mol_type = other DNA
tgagagtgcaccatatgaagcttgggaatgccgatgtcg

SEQ ID NO: 12 - DNA, 18 bp, synthetic construct
  source 1..18: mol_type = other DNA
attccgaccagcgaagtg

SEQ ID NO: 13 - DNA, 37 bp, synthetic construct
  source 1..37: mol_type = other DNA
cacttcgctggtcggaatatgaacatgtctctgtcac

SEQ ID NO: 14 - DNA, 42 bp, synthetic construct
  source 1..42: mol_type = other DNA
cgtcccgttctcggtcaaggcatttaccagctgtaccggtag

SEQ ID NO: 15 - DNA, 30 bp, synthetic construct
  source 1..30: mol_type = other DNA
cgagttcttctgacattccaccatcgagag

SEQ ID NO: 16 - DNA, 34 bp, synthetic construct
  source 1..34: mol_type = other DNA
gctcacatgtggatcccctcggcagccttgacca

SEQ ID NO: 17 - DNA, 64 bp, synthetic construct
  source 1..64: mol_type = other DNA
accgagaacgggacggtcaccatatcggccgattcggccgtgctcgagccggaattgccagctg

SEQ ID NO: 18 - DNA, 29 bp, synthetic construct
  source 1..29: mol_type = other DNA
gtggaatgtcagaagaactcgtcaagaag

SEQ ID NO: 19 - DNA, 29 bp, synthetic construct
  source 1..29: mol_type = other DNA
gtggaatgtcagaagaactcgtcaagaag

SEQ ID NO: 20 - DNA, 38 bp, synthetic construct
  source 1..38: mol_type = other DNA
ggccgattcggccgtgctcgagccggaattgccagctg

SEQ ID NO: 21 - DNA, 20 bp, synthetic construct
  source 1..20: mol_type = other DNA
gatgtccttgttggacatgc

SEQ ID NO: 22 - DNA, 26 bp, synthetic construct
  source 1..26: mol_type = other DNA
attccggctcgagcacggccgaatcg

SEQ ID NO: 23 - DNA, 27 bp, synthetic construct
  source 1..27: mol_type = other DNA
tcgtacgagtactccaagggcccgaag

SEQ ID NO: 24 - DNA, 26 bp, synthetic construct
  source 1..26: mol_type = other DNA
gcgaatcttgttggagaaacgggtgt

SEQ ID NO: 25 - DNA, 25 bp, synthetic construct
  source 1..25: mol_type = other DNA
cctgatgttggcgtgtacgggtctt

SEQ ID NO: 26 - DNA, 23 bp, synthetic construct
  source 1..23: mol_type = other DNA
gatcgtgacggtgccctgttgga